European Patent Application EP 4 321 537 A1, published February 14, 2024. Title: 药物组合物及其用途. Applicant: 中山康方生物医药有限公司. The sequence listing filed with the application follows.

SEQUENCE LISTING (48 sequences)

SEQ ID NO: 1 - DNA, 363 bp, synthetic construct
  source 1..363: mol_type = other DNA
gaggtgcagctgcagcagtccggaccagagctggtgaagcctggcgcctccatgcggatgtcttgtaaggcctctggctacagcttcaccggctatacaatgaactgggtgaagcagtctcacggcaagaatctggagtggatcggcctgatcaacccttacaatgccggcaccagctataaccagaagtttaagggcaaggccaccctgacagtggacaagagctcctctaccgcctacatggagctgctgtccctgacatctgaggatagcgccgtgtactattgcgcccggtccgagtacagatatggcggcgactactttgattattggggccagggcaccacactgacagtgagctcc

SEQ ID NO: 2 - protein, 121 aa, synthetic construct
EVQLQQSGPELVKPGASMRMSCKASGYSFTGYTMNWVKQSHGKNLEWIGLINPYNAGTSYNQKFKGKATLTVDKSSSTAYMELLSLTSEDSAVYYCARSEYRYGGDYFDYWGQGTTLTVSS

SEQ ID NO: 3 - DNA, 339 bp, synthetic construct
  source 1..339: mol_type = other DNA
gacatcgtgatgacccagtctccaagctccctggcaatgagcgtgggacagaaggtgacaatgtcttgtaagtctagccagagcctgctgaactcctctaatcagaagaactacctggcctggtatcagcagaagccaggccagtctcccaagctgctggtgtactttgccagcaccagggagtccggagtgcctgacagattcatcggctccggctctggcacagacttcaccctgacaatcagctccgtgcaggcagaggacctggcagattatttctgccagcagcactacgacaccccttatacatttggcggcggcaccaagctggagatcaag

SEQ ID NO: 4 - protein, 113 aa, synthetic construct
DIVMTQSPSSLAMSVGQKVTMSCKSSQSLLNSSNQKNYLAWYQQKPGQSPKLLVYFASTRESGVPDRFIGSGSGTDFTLTISSVQAEDLADYFCQQHYDTPYTFGGGTKLEIK

SEQ ID NO: 5 - DNA, 363 bp, synthetic construct
  source 1..363: mol_type = other DNA
caggtgcagctgcagcagtctggagcagaggtggtgaagccaggagcctctatgaagatgagctgtaaggccagcggctactccttcaccggctatacaatgaactgggtgaagcaggcccacggccagaatctggagtggatcggcctgatcaacccttacaatgccggcacctcttataaccagaagtttcagggcaaggccaccctgacagtggacaagtccacctctacagcctacatggagctgagctccctgcggagcgaggatacagccgtgtactattgcgcccggtccgagtacagatatggcggcgactactttgattattggggccagggcaccacactgaccgtgtctagc

SEQ ID NO: 6 - protein, 121 aa, synthetic construct
QVQLQQSGAEVVKPGASMKMSCKASGYSFTGYTMNWVKQAHGQNLEWIGLINPYNAGTSYNQKFQGKATLTVDKSTSTAYMELSSLRSEDTAVYYCARSEYRYGGDYFDYWGQGTTLTVSS

SEQ ID NO: 7 - DNA, 339 bp, synthetic construct
  source 1..339: mol_type = other DNA
gacatcgtgatgacccagtccccaagctccctggcaatgtctgtgggagagagggtgacaatgtcctgtaagtctagccagtctctgctgaactcctctaatcagaagaactacctggcctggtatcagcagaagcccggccaggcccctaagctgctggtgtactttgcctctaccagggagagcggagtgccagacagattctctggcagcggctccggcacagacttcaccctgacaatcagctccgtgcaggcagaggacctggcagattatttctgccagcagcactacgataccccctatacatttggcggcggcaccaagctggagatcaag

SEQ ID NO: 8 - protein, 113 aa, synthetic construct
DIVMTQSPSSLAMSVGERVTMSCKSSQSLLNSSNQKNYLAWYQQKPGQAPKLLVYFASTRESGVPDRFSGSGSGTDFTLTISSVQAEDLADYFCQQHYDTPYTFGGGTKLEIK

SEQ ID NO: 9 - DNA, 363 bp, synthetic construct
  source 1..363: mol_type = other DNA
caggtgcagctggtgcagtctggagcagaggtggtgaagccaggagcctctgtgaaggtgagctgtaaggccagcggctactccttcaccggctatacaatgaactgggtgaggcaggcaccaggacagaatctggagtggatcggcctgatcaacccttacaatgccggcacctcttataaccagaagtttcagggcaaggtgaccctgacagtggacaagtccacctctacagcctacatggagctgagctccctgcggagcgaggatacagccgtgtactattgcgcccggtccgagtacagatatggcggcgactactttgattattggggccagggcaccacactgaccgtgtctagc

SEQ ID NO: 10 - protein, 121 aa, synthetic construct
QVQLVQSGAEVVKPGASVKVSCKASGYSFTGYTMNWVRQAPGQNLEWIGLINPYNAGTSYNQKFQGKVTLTVDKSTSTAYMELSSLRSEDTAVYYCARSEYRYGGDYFDYWGQGTTLTVSS

SEQ ID NO: 11 - DNA, 339 bp, synthetic construct
  source 1..339: mol_type = other DNA
gacatcgtgatgacccagtccccaagctccctggccgtgtctgtgggagagcgggtgacaatctcctgtaagtctagccagtctctgctgaactcctctaatcagaagaactacctggcctggtatcagcagaagcccggccaggcccctaagctgctgatctacttcgcctctaccagggagagcggagtgccagacagattctctggcagcggctccggcacagacttcaccctgacaatcagctccgtgcaggcagaggacgtggcagattactattgccagcagcactacgataccccctatacatttggcggcggcaccaagctggagatcaag

SEQ ID NO: 12 - protein, 113 aa, synthetic construct
DIVMTQSPSSLAVSVGERVTISCKSSQSLLNSSNQKNYLAWYQQKPGQAPKLLIYFASTRESGVPDRFSGSGSGTDFTLTISSVQAEDVADYYCQQHYDTPYTFGGGTKLEIK

SEQ ID NO: 13 - DNA, 339 bp, synthetic construct
  source 1..339: mol_type = other DNA
gacatcgtgatgacccagtccccaagctccctggccgtgtctgtgggagagcgggtgacaatctcctgtaagtctagccagtctctgctgaactcctctaatcagaagaactacctggcctggtatcagcagaagcccggccaggcccctaagctgctgatctacttcgcctctaccagggagagcggagtgccagacagattctctggcagcggctccggcacagacttcaccctgacaatcagctccctgcaggcagaggacgtggccgtgtactattgccagcagcactacgataccccctatacatttggcggcggcaccaagctggagatcaag

SEQ ID NO: 14 - protein, 113 aa, synthetic construct
DIVMTQSPSSLAVSVGERVTISCKSSQSLLNSSNQKNYLAWYQQKPGQAPKLLIYFASTRESGVPDRFSGSGSGTDFTLTISSLQAEDVAVYYCQQHYDTPYTFGGGTKLEIK

SEQ ID NO: 15 - protein, 8 aa, synthetic construct
GYSFTGYT

SEQ ID NO: 16 - protein, 8 aa, synthetic construct
INPYNAGT

SEQ ID NO: 17 - protein, 14 aa, synthetic construct
ARSEYRYGGDYFDY

SEQ ID NO: 18 - protein, 12 aa, synthetic construct
QSLLNSSNQKNY

SEQ ID NO: 19 - skipped

SEQ ID NO: 20 - protein, 9 aa, synthetic construct
QQHYDTPYT

SEQ ID NO: 21 - protein, 330 aa, synthetic construct
ASTKGPSVFPLAPSSKSTSGGTAALGCLVKDYFPEPVTVSWNSGALTSGVHTFPAVLQSSGLYSLSSVVTVPSSSLGTQTYICNVNHKPSNTKVDKKVEPKSCDKTHTCPPCPAPEAAGGPSVFLFPPKPKDTLMISRTPEVTCVVVDVSHEDPEVKFNWYVDGVEVHNAKTKPREEQYNSTYRVVSVLTVLHQDWLNGKEYKCKVSNKALPAPIEKTISKAKGQPREPQVYTLPPSRDELTKNQVSLTCLVKGFYPSDIAVEWESNGQPENNYKTTPPVLDSDGSFFLYSKLTVDKSRWQQGNVFSCSVMHEALHNHYTQKSLSLSPGK

SEQ ID NO: 22 - protein, 107 aa, synthetic construct [sequence omitted]

SEQ ID NO: 23 - protein, 719 aa, synthetic construct
EVQLVESGGGLVQPGGSLRLSCAASGYTFTNYGMNWVRQAPGKGLEWVGWINTYTGEPTYAADFKRRFTFSLDTSKSTAYLQMNSLRAEDTAVYYCAKYPHYYGSSHWYFDVWGQGTLVTVSSASTKGPSVFPLAPSSKSTSGGTAALGCLVKDYFPEPVTVSWNSGALTSGVHTFPAVLQSSGLYSLSSVVTVPSSSLGTQTYICNVNHKPSNTKVDKKVEPKSCDKTHTCPPCPAPEAAGGPSVFLFPPKPKDTLMISRTPEVTCVVVDVSHEDPEVKFNWYVDGVEVHNAKTKPREEQYNSTYRVVSVLTVLHQDWLNGKEYKCKVSNKALPAPIEKTISKAKGQPREPQVYTLPPSRDELTKNQVSLTCLVKGFYPSDIAVEWESNGQPENNYKTTPPVLDSDGSFFLYSKLTVDKSRWQQGNVFSCSVMHEALHNHYTQKSLSLSPGKGGGGSGGGGSGGGGSGGGGSEVQLVESGGGLVQPGGSLRLSCAASGFAFSSYDMSWVRQAPGKGLDWVATISGGGRYTYYPDSVKGRFTISRDNSKNNLYLQMNSLRAEDTALYYCANRYGEAWFAYWGQGTLVTVSSGGGGSGGGGSGGGGSGGGGSDIQMTQSPSSMSASVGDRVTFTCRASQDINTYLSWFQQKPGKSPKTLIYRANRLVSGVPSRFSGSGSGQDYTLTISSLQPEDMATYYCLQYDEFPLTFGAGTKLELKR

SEQ ID NO: 24 - DNA, 2157 bp, synthetic construct
  source 1..2157: mol_type = other DNA
gaggtgcagctggtcgagtccgggggggggctggtgcagccaggcgggtctctgaggctgagttgcgccgcttcagggtacaccttcacaaactatggaatgaattgggtgcgccaggcaccaggaaagggactggagtgggtcggctggatcaacacttacaccggggaacctacctatgcagccgactttaagcggcggttcaccttcagcctggatacaagcaaatccactgcctacctgcagatgaacagcctgcgagctgaggacaccgcagtctactattgtgctaaatatccccactactatgggagcagccattggtattttgacgtgtgggggcaggggactctggtgacagtgagcagcgcaagcaccaaagggcccagcgtgtttcctctcgccccctcctccaaaagcaccagcggaggaaccgctgctctcggatgtctggtgaaggactacttccctgaacccgtcaccgtgagctggaatagcggcgctctgacaagcggagtccatacattccctgctgtgctgcaaagcagcggactctattccctgtccagcgtcgtcacagtgcccagcagcagcctgggcacccagacctacatctgtaacgtcaaccacaagccctccaacaccaaggtggacaagaaagtggagcccaaatcctgcgacaagacacacacctgtcccccctgtcctgctcccgaagctgctggaggccctagcgtcttcctctttcctcccaaacccaaggacaccctcatgatcagcagaacccctgaagtcacctgtgtcgtcgtggatgtcagccatgaggaccccgaggtgaaattcaactggtatgtcgatggcgtcgaggtgcacaacgccaaaaccaagcccagggaggaacagtacaactccacctacagggtggtgtccgtgctgacagtcctccaccaggactggctgaacggcaaggagtacaagtgcaaggtgtccaacaaggctctccctgcccccattgagaagaccatcagcaaggccaaaggccaacccagggagccccaggtctatacactgcctccctccagggacgaactcaccaagaaccaggtgtccctgacctgcctggtcaagggcttttatcccagcgacatcgccgtcgagtgggagtccaacggacagcccgagaataactacaagaccacccctcctgtcctcgactccgacggctccttcttcctgtacagcaaactgaccgtcgataaatctaggtggcagcagggcaacgtgttctcttgttccgtgatgcatgaagcactgcacaaccattatacccagaagtctctgagcctgtcccccggcaagggcggcggcggctctggaggaggaggcagcggcggaggaggctccggaggcggcggctctgaggtgcagctggtggagtctggaggaggactggtgcagcctggaggctccctgaggctgtcttgcgcagcaagcggattcgcctttagctcctacgacatgagctgggtgcggcaggcacctggcaagggtctggattgggtggcaaccatcagcggaggcggcagatacacatactatcccgactccgtgaagggcaggttcaccatctcccgcgataactctaagaacaatctgtatctgcagatgaacagcctgagggccgaggacacagccctgtactattgcgccaaccgctacggcgaggcctggtttgcctattggggccagggcaccctggtgacagtgtctagcggcggcggcggcagcggcggcggcggctccggaggaggcggctctggcggcggcggcagcgatatccagatgacccagtccccctcctctatgtctgccagcgtgggcgaccgggtgaccttcacatgtagagcctcccaggatatcaacacctacctgtcttggtttcagcagaagcccggcaagagccctaagacactgatctatcgggccaatagactggtgagcggagtgccttcccggttctccggctctggcagcggacaggactataccctgacaatcagctccctgcagccagaggatatggccacatactattgcctgcagtatgacgagttccccctgaccttcggggctggcactaagctggagctgaaaaga

SEQ ID NO: 25 - protein, 214 aa, synthetic construct
DIQMTQSPSSLSASVGDRVTITCSASQDISNYLNWYQQKPGKAPKVLIYFTSSLHSGVPSRFSGSGSGTDFTLTISSLQPEDFATYYCQQYSTVPWTFGQGTKVEIKRTVAAPSVFIFPPSDEQLKSGTASVVCLLNNFYPREAKVQWKVDNALQSGNSQESVTEQDSKDSTYSLSSTLTLSKADYEKHKVYACEVTHQGLSSPVTKSFNRGEC

SEQ ID NO: 26 - DNA, 642 bp, synthetic construct
  source 1..642: mol_type = other DNA
gatattcagatgactcagagcccctcctccctgtccgcctctgtgggcgacagggtcaccatcacatgcagtgcttcacaggatatttccaactacctgaattggtatcagcagaagccaggaaaagcacccaaggtgctgatctacttcactagctccctgcactcaggagtgccaagccggttcagcggatccggatctggaaccgactttactctgaccatttctagtctgcagcctgaggatttcgctacatactattgccagcagtattctaccgtgccatggacatttggccaggggactaaagtcgagatcaagcggaccgtggccgctcccagtgtcttcatttttccccctagcgacgaacagctgaaatccgggacagcctctgtggtctgtctgctgaacaacttctaccctagagaggcaaaagtgcagtggaaggtcgataacgccctgcagagtggcaattcacaggagagcgtgacagaacaggactccaaagattctacttatagtctgtcaagcacactgactctgagcaaggctgactacgaaaagcataaagtgtatgcatgtgaggtcacccaccaggggctgagcagtccagtcaccaagtcattcaacagaggcgagtgc

SEQ ID NO: 27 - protein, 123 aa, synthetic construct [sequence omitted]

SEQ ID NO: 28 - DNA, 369 bp, synthetic construct
  source 1..369: mol_type = other DNA
gaggtgcagctggtcgagtccgggggggggctggtgcagccaggcgggtctctgaggctgagttgcgccgcttcagggtacaccttcacaaactatggaatgaattgggtgcgccaggcaccaggaaagggactggagtgggtcggctggatcaacacttacaccggggaacctacctatgcagccgactttaagcggcggttcaccttcagcctggatacaagcaaatccactgcctacctgcagatgaacagcctgcgagctgaggacaccgcagtctactattgtgctaaatatccccactactatgggagcagccattggtattttgacgtgtgggggcaggggactctggtgacagtgagcagc

SEQ ID NO: 29 - protein, 107 aa, synthetic construct [sequence omitted]

SEQ ID NO: 30 - DNA, 321 bp, synthetic construct
  source 1..321: mol_type = other DNA
gatattcagatgactcagagcccctcctccctgtccgcctctgtgggcgacagggtcaccatcacatgcagtgcttcacaggatatttccaactacctgaattggtatcagcagaagccaggaaaagcacccaaggtgctgatctacttcactagctccctgcactcaggagtgccaagccggttcagcggatccggatctggaaccgactttactctgaccatttctagtctgcagcctgaggatttcgctacatactattgccagcagtattctaccgtgccatggacatttggccaggggactaaagtcgagatcaag

SEQ ID NO: 31 - protein, 8 aa, synthetic construct
GYTFTNYG

SEQ ID NO: 32 - protein, 8 aa, synthetic construct
INTYTGEP

SEQ ID NO: 33 - protein, 16 aa, synthetic construct
AKYPHYYGSSHWYFDV

SEQ ID NO: 34 - protein, 6 aa, synthetic construct
QDISNY

SEQ ID NO: 35 - skipped

SEQ ID NO: 36 - protein, 9 aa, synthetic construct
QQYSTVPWT

SEQ ID NO: 37 - protein, 118 aa, synthetic construct
EVQLVESGGGLVQPGGSLRLSCAASGFAFSSYDMSWVRQAPGKGLDWVATISGGGRYTYYPDSVKGRFTISRDNSKNNLYLQMNSLRAEDTALYYCANRYGEAWFAYWGQGTLVTVSS

SEQ ID NO: 38 - DNA, 354 bp, synthetic construct
  source 1..354: mol_type = other DNA
gaagtgcagctggtcgagtctgggggagggctggtgcagcccggcgggtcactgcgactgagctgcgcagcttccggattcgcctttagctcctacgacatgtcctgggtgcgacaggcaccaggaaagggactggattgggtcgctactatctcaggaggcgggagatacacctactatcctgacagcgtcaagggccggttcacaatctctagagataacagtaagaacaatctgtatctgcagatgaacagcctgagggctgaggacaccgcactgtactattgtgccaaccgctacggggaagcatggtttgcctattgggggcagggaaccctggtgacagtctctagt

SEQ ID NO: 39 - protein, 108 aa, synthetic construct
DIQMTQSPSSMSASVGDRVTFTCRASQDINTYLSWFQQKPGKSPKTLIYRANRLVSGVPSRFSGSGSGQDYTLTISSLQPEDMATYYCLQYDEFPLTFGAGTKLELKR

SEQ ID NO: 40 - DNA, 324 bp, synthetic construct
  source 1..324: mol_type = other DNA
gatatccagatgacccagtccccctcctctatgtctgccagcgtgggcgaccgggtgaccttcacatgtagagcctcccaggatatcaacacctacctgtcttggtttcagcagaagcccggcaagagccctaagacactgatctatcgggccaatagactggtgagcggagtgccttcccggttctccggctctggcagcggacaggactataccctgacaatcagctccctgcagccagaggatatggccacatactattgcctgcagtatgacgagttccccctgaccttcggggctggcactaagctggagctgaaaaga

SEQ ID NO: 41 - protein, 8 aa, synthetic construct
GFAFSSYD

SEQ ID NO: 42 - protein, 8 aa, synthetic construct
ISGGGRYT

SEQ ID NO: 43 - protein, 11 aa, synthetic construct
ANRYGEAWFAY

SEQ ID NO: 44 - protein, 6 aa, synthetic construct
QDINTY

SEQ ID NO: 45 - skipped

SEQ ID NO: 46 - protein, 9 aa, synthetic construct
LQYDEFPLT

SEQ ID NO: 47 - protein, 15 aa, synthetic construct
GGGGSGGGGSGGGGS

SEQ ID NO: 48 - protein, 20 aa, synthetic construct
GGGGSGGGGSGGGGSGGGGS